European Patent Specification EP 4 034 155 B1, published May 14, 2025. Title: MULTI-ANTIGENIC PEPTIDE MIMICS OF GONOCOCCAL LIPO-OLIGOSACCHARIDE (LOS) EPITOPES. Applicant: UNIVERSITY OF MASSACHUSETTS. Application Not Yet Assigned. The sequence listing filed with the application follows.

SEQUENCE LISTING (19 sequences)

SEQ ID NO: 1 - protein, 17 aa, Artificial Sequence
  Synthetic
GPIPVLDENGLFAPGPC

SEQ ID NO: 2 - protein, 12 aa, Artificial Sequence
  Synthetic
IPVLDENGLFAP

SEQ ID NO: 3 - protein, 13 aa, Artificial Sequence
  Synthetic
KIPVLDENGLFAP

SEQ ID NO: 4 - protein, 28 aa, Artificial Sequence
  Synthetic
KIPVLDENGLFAPGSKIPVLDENGLFAP

SEQ ID NO: 5 - protein, 5 aa, Artificial Sequence
  Synthetic
AAAGG

SEQ ID NO: 6 - protein, 31 aa, Artificial Sequence
  Synthetic
KIPVLDENGLFAPAAAGGKIPVLDENGLFAP

SEQ ID NO: 7 - protein, 18 aa, Artificial Sequence
  Synthetic
GPIPVLDENGLFAPGPCK

SEQ ID NO: 8 - protein, 18 aa, Artificial Sequence
  Synthetic
CGPIPVLDENGLFAPGPC

SEQ ID NO: 9 - protein, 18 aa, Artificial Sequence
  Synthetic
SGPIPVLDENGLFAPGPS

SEQ ID NO: 10 - protein, 16 aa, Artificial Sequence
  Synthetic
KIPVLDENGLFAPGPC

SEQ ID NO: 11 - protein, 15 aa, Artificial Sequence
  Synthetic
SGPIPVLDENGLFAP

SEQ ID NO: 12 - protein, 18 aa, Artificial Sequence
  Synthetic
AGPIPVLDENGLFAPGPC

SEQ ID NO: 13 - protein, 14 aa, Artificial Sequence
  Synthetic
CIPVLDENGLFAPC

SEQ ID NO: 14 - protein, 19 aa, Artificial Sequence
  Synthetic
CGPPEARDEGTITLERGPC

SEQ ID NO: 15 - protein, 18 aa, Artificial Sequence
  Synthetic
SGPIPVLDENGLFAPGPC

SEQ ID NO: 16 - protein, 29 aa, Artificial Sequence
  Synthetic
KIPVLDENGLFAPGSKKIPVLDENGLFAP

SEQ ID NO: 17 - protein, 19 aa, Artificial Sequence
  Synthetic
GPCIPVLDENGLFAPCGPK

SEQ ID NO: 18 - protein, 19 aa, Artificial Sequence
  Synthetic
CGPIPVLDENGLFAPGPCK

SEQ ID NO: 19 - protein, 18 aa, Artificial Sequence
  Synthetic
CPGPAFLGNEDLVPIPFC